European Patent Application EP 4 400 581 A1, published July 17, 2024. Title: A method for producing pluripotent stem cell-derived hematopoietic stem cells and a method for producing a humanized mouse model using the prepared hematopoietic stem cells. Applicant: SUNGKWANG MEDICAL FOUNDATION. The sequence listing filed with the application follows.

SEQUENCE LISTING (2 sequences)

SEQ ID NO: 1 - DNA, 22 bp, synthetic construct
  source 1..22: mol_type = other DNA
caacactaaaggacgaacctga

SEQ ID NO: 2 - DNA, 20 bp, synthetic construct
  source 1..20: mol_type = other DNA
tcgtaaggggtggatttttc